European Patent Application EP 4 446 433 A1, published October 16, 2024. Title: Digital Amplification Detection Method for Simultaneously Identifying Multiple Genotypes, Detection Product and Detection Kit. Applicant: NANJING PREGENE BIOTECHNOLOGY Co.,Ltd. Application IB PCT/CN2022/120663, filed September 22, 2022. The sequence listing filed with the application follows.

SEQUENCE LISTING (35 sequences)

SEQ ID NO: 1 - DNA, 18 bp, synthetic construct
  source 1..18: mol_type = other DNA
ccgccgcggccgccgcct

SEQ ID NO: 2 - DNA, 17 bp, synthetic construct
  source 1..17: mol_type = other DNA
cgccgccgcgtccgcgc

SEQ ID NO: 3 - DNA, 15 bp, synthetic construct
  source 1..15: mol_type = other DNA
cccgcccctccgggg

SEQ ID NO: 4 - DNA, 15 bp, synthetic construct
  source 1..15: mol_type = other DNA
ccggggcgccgcggg

SEQ ID NO: 5 - DNA, 20 bp, synthetic construct
  source 1..20: mol_type = other DNA
tgccgccgccgctgctgcct

SEQ ID NO: 6 - DNA, 14 bp, synthetic construct
  source 1..14: mol_type = other DNA
cgccaccttcgccg

SEQ ID NO: 7 - DNA, 13 bp, synthetic construct
  source 1..13: mol_type = other DNA
gtacctctctccc

SEQ ID NO: 8 - DNA, 10 bp, synthetic construct
  source 1..10: mol_type = other DNA
ggaagcagca

SEQ ID NO: 9 - DNA, 27 bp, synthetic construct
  source 1..27: mol_type = other DNA
ccctgggggagtattgcggaggaaggg

SEQ ID NO: 10 - DNA, 13 bp, synthetic construct
  source 1..13: mol_type = other DNA
acataaaaaaata

SEQ ID NO: 11 - DNA, 17 bp, synthetic construct
  source 1..17: mol_type = other DNA
aaaaattcaatttctaa

SEQ ID NO: 12 - DNA, 14 bp, synthetic construct
  source 1..14: mol_type = other DNA
aaatattttataat

SEQ ID NO: 13 - DNA, 28 bp, synthetic construct
  source 1..28: mol_type = other DNA
aacttcaaaacaaacaaaacaaaacaca

SEQ ID NO: 14 - DNA, 12 bp, synthetic construct
  source 1..12: mol_type = other DNA
tgagataacctg

SEQ ID NO: 15 - DNA, 15 bp, synthetic construct
  source 1..15: mol_type = other DNA
gcagtagaaataatc

SEQ ID NO: 16 - DNA, 20 bp, synthetic construct
  source 1..20: mol_type = other DNA
gatagtaataccactctgtc

SEQ ID NO: 17 - DNA, 24 bp, synthetic construct
  source 1..24: mol_type = other DNA
ttcagattagaataccatttctta

SEQ ID NO: 18 - DNA, 16 bp, synthetic construct
  source 1..16: mol_type = other DNA
cacataaacaaatttt

SEQ ID NO: 19 - DNA, 17 bp, synthetic construct
  source 1..17: mol_type = other DNA
ataattaaaaatttcca

SEQ ID NO: 20 - DNA, 10 bp, synthetic construct
  source 1..10: mol_type = other DNA
acacggtatt

SEQ ID NO: 21 - DNA, 130 bp, synthetic construct
  source 1..130: mol_type = other DNA
tcctcatctgtcgagactcactataggaagagatgtcaactcgtgcacgagttgacatctcttctccgagccggtcgaaatattggaggaagctcgagctggaggaaaagtgagtctcgacagatgagga

SEQ ID NO: 22 - DNA, 126 bp, synthetic construct
  source 1..126: mol_type = other DNA
actcatctgtgagactcactataggaagagatgtcaactcgtgcacgagttgacatctcttctccgagccggtcgaaatattggaggaagctcgagctggaggaaaagtgagtctcacagatgagt

SEQ ID NO: 23 - DNA, 21 bp, synthetic construct
  source 1..21: mol_type = other DNA
tgggtgacagagtgagacttc

SEQ ID NO: 24 - DNA, 20 bp, synthetic construct
  source 1..20: mol_type = other DNA
acccggccctcattatttct

SEQ ID NO: 25 - DNA, 20 bp, synthetic construct
  source 1..20: mol_type = other DNA
ccaacatggtgaaaccccaa

SEQ ID NO: 26 - DNA, 19 bp, synthetic construct
  source 1..19: mol_type = other DNA
ccgaagtgctgggattaca

SEQ ID NO: 27 - DNA, 20 bp, synthetic construct
  source 1..20: mol_type = other DNA
ggcacctctaatcccagcta

SEQ ID NO: 28 - DNA, 18 bp, synthetic construct
  source 1..18: mol_type = other DNA
cctcagcctcccgaagtg

SEQ ID NO: 29 - DNA, 22 bp, synthetic construct
  source 1..22: mol_type = other DNA
acgttgataccatactggaggt

SEQ ID NO: 30 - DNA, 15 bp, synthetic construct
  source 1..15: mol_type = other DNA
aggatttgactctca

SEQ ID NO: 31 - DNA, 25 bp, synthetic construct
  source 1..25: mol_type = other DNA
tactcaggaggctgaggcaggagaa

SEQ ID NO: 32 - DNA, 25 bp, synthetic construct
  source 1..25: mol_type = other DNA
ttgcttggacctgggaggcagaggt

SEQ ID NO: 33 - DNA, 21 bp, synthetic construct
  source 1..21: mol_type = other DNA
ggaggcagaggttgcagtgag

SEQ ID NO: 34 - DNA, 20 bp, synthetic construct
  source 1..20: mol_type = other DNA
gagatcgcgctattgcactc

SEQ ID NO: 35 - DNA, 133 bp, synthetic construct
  source 1..133: mol_type = other DNA
aatgccaacaatgaccgcaggtacccagattcaaggagaacagaagcagtcagtcatggccccctggtgtttttgaataatttgggtaaaaagaagggacggactgaagatggaggtacgagattgttggcac